European Patent Specification EP 3 538 131 B1, published May 7, 2025. Title: MANP ANALOGUES. Applicant: Mayo Foundation for Medical Education and Research. The sequence listing filed with the application follows.

SEQUENCE LISTING (15 sequences)

SEQ ID NO: 1 - protein, 40 aa, Homo sapiens
SLRRSSCFGGRMDRIGAQSGLGCNSFRYRITAREDKQGWA

SEQ ID NO: 2 - protein, 44 aa, Artificial Sequence
  synthetic
TAPRSLRRSSCFGGRMDRIGAQSGLGCNSFRYRITAREDKQGWA

SEQ ID NO: 3 - protein, 40 aa, Artificial Sequence
  synthetic
SLKKSSCFGGRMDRIGAQSGLGCNSFRYRITAREDKQGWA

SEQ ID NO: 4 - protein, 40 aa, Artificial Sequence; identical to SEQ ID NO: 1
  synthetic
  MISC_FEATURE (6)..(6): D-form

SEQ ID NO: 5 - protein, 39 aa, Artificial Sequence
  synthetic
  MISC_FEATURE (4)..(4): D-form
SLRRSCFGGRMDRIGAQSGLGCNSFRYRITAREDKQGWA

SEQ ID NO: 6 - protein, 40 aa, Artificial Sequence
  synthetic
TLRRTTCFGGRMDRIGAQSGLGCNSFRYRITAREDKQGWA

SEQ ID NO: 7 - protein, 28 aa, Homo sapiens
SLRRSSCFGGRMDRIGAQSGLGCNSFRY

SEQ ID NO: 8 - protein, 32 aa, Homo sapiens
SPKMVQGSGCFGRKMDRISSSSGLGCKVLRRH

SEQ ID NO: 9 - protein, 22 aa, Homo sapiens
GLSKGCFGLKLDRIGSMSGLGC

SEQ ID NO: 10 - protein, 32 aa, Homo sapiens
TAPRSLRRSSCFGGRMDRIGAQSGLGCNSFRY

SEQ ID NO: 11 - protein, 38 aa, Dendroaspis angusticeps
EVKYDPCFGHKIDRINHVSNLGCPSLRDPRPNAPSTSA

SEQ ID NO: 12 - protein, 12 aa, Homo sapiens
RITAREDKQGWA

SEQ ID NO: 13 - DNA, 93 bp, Homo sapiens
agcctgcggagatccagctgcttcgggggcaggatggacaggattggagcccagagcggactgggctgtaacagcttccggtaccgaagataa

SEQ ID NO: 14 - DNA, 123 bp, Homo sapiens
agcctgcggagatccagctgcttcgggggcaggatggacaggattggagcccagagcggactgggctgtaacagcttccggtaccggataacagccagggaggacaagcagggctgggcctag

SEQ ID NO: 15 - protein, 41 aa, Artificial Sequence
  synthetic
SWLRRSSCFGGRMDRIGAQSGLGCNSFRYRITAREDKQGWA